European Patent Application EP 4 609 882 A1, published September 3, 2025. Title: 遺伝子導入法、遺伝子治療法、および組織再生法. Applicant: 栗田　昌和. Application WO. The sequence listing filed with the application follows.

SEQUENCE LISTING (31 sequences)

SEQ ID NO: 1 - protein, 11 aa, synthetic construct
QRGXXXXXXXA

SEQ ID NO: 2 - protein, 7 aa, synthetic construct
EPKARAP

SEQ ID NO: 3 - protein, 737 aa, synthetic construct
MAADGYLPDWLEDTLSEGIRQWWKLKPGPPPPKPAERHKDDSRGLVLPGYKYLGPFNGLDKGEPVNEADAAALEHDKAYDRQLDSGDNPYLKYNHADAEFQERLKEDTSFGGNLGRAVFQAKKRLLEPLGLVEEAAKTAPGKKRPVEHSPVEPDSSSGTGKAGQQPARKRLNFGQTGDADSVPDPQPIGEPPAAPSGVGSLTMAAGGGAPMADNNEGADGVGNSSGNWHCDSTWMGDRVITTSTRTWALPTYNNHLYKQISNSTSGGSSNDNAYFGYSTPWGYFDFNRFHCHFSPRDWQRLINNNWGFRPKRLSFKLFNIQVKEVTQNEGTKTIANNLTSTIQVFTDSEYQLPYVLGSAHQGCLPPFPADVFMIPQYGYLTLNNGSQAVGRSSFYCLEYFPSQMLRTGNNFQFTYTFEDVPFHSSYAHSQSLDRLMNPLIDQYLYYLSRTQTTGGTTNTQTLGFSQGGPNTMANQAKNWLPGPCYRQQRVSKTSADNNNSEYSWTGATKYHLNGRDSLVNPGPAMASHKDDEEKFFPQSGVLIFGKQGSEKTNVDIEKVMITDEEEIRTTNPVATEQYGSVSTNLQRGNRQAATADVNTQGVLPGMVWQDRDVYLQGPIWAKIPHTDGHFHPSPLMGGFGLKHPPPQILIKNTPVPADPPTTFNQSKLNSFITQYSTGQVSVEIEWELQKENSKRWNPEIQYTSNYYKSTSVDFAVNTEGVYSEPRPIGTRYLTRNL

SEQ ID NO: 4 - protein, 11 aa, synthetic construct
QRGEPKARAPA

SEQ ID NO: 5 - protein, 746 aa, synthetic construct
MAADGYLPDWLEDTLSEGIRQWWKLKPGPPPPKPAERHKDDSRGLVLPGYKYLGPFNGLDKGEPVNEADAAALEHDKAYDRQLDSGDNPYLKYNHADAEFQERLKEDTSFGGNLGRAVFQAKKRLLEPLGLVEEAAKTAPGKKRPVEHSPVEPDSSSGTGKAGQQPARKRLNFGQTGDADSVPDPQPIGEPPAAPSGVGSLTMAAGGGAPMADNNEGADGVGNSSGNWHCDSTWMGDRVITTSTRTWALPTYNNHLYKQISNSTSGGSSNDNAYFGYSTPWGYFDFNRFHCHFSPRDWQRLINNNWGFRPKRLSFKLFNIQVKEVTQNEGTKTIANNLTSTIQVFTDSEYQLPYVLGSAHQGCLPPFPADVFMIPQYGYLTLNNGSQAVGRSSFYCLEYFPSQMLRTGNNFQFTYTFEDVPFHSSYAHSQSLDRLMNPLIDQYLYYLSRTQTTGGTTNTQTLGFSQGGPNTMANQAKNWLPGPCYRQQRVSKTSADNNNSEYSWTGATKYHLNGRDSLVNPGPAMASHKDDEEKFFPQSGVLIFGKQGSEKTNVDIEKVMITDEEEIRTTNPVATEQYGSVSTNLQRGQRGEPKARAPAQAATADVNTQGVLPGMVWQDRDVYLQGPIWAKIPHTDGHFHPSPLMGGFGLKHPPPQILIKNTPVPADPPTTFNQSKLNSFITQYSTGQVSVEIEWELQKENSKRWNPEIQYTSNYYKSTSVDFAVNTEGVYSEPRPIGTRYLTRNL

SEQ ID NO: 6 - DNA, 2241 bp, synthetic construct
  source 1..2241: mol_type = other DNA
atggctgccgatggttatcttccagattggctcgaggacactctctctgaaggaataagacagtggtggaagctcaaacctggcccaccaccaccaaagcccgcagagcggcataaggacgacagcaggggtcttgtgcttcctgggtacaagtacctcggacccttcaacggactcgacaagggagagccggtcaacgaggcagacgccgcggccctcgagcacgacaaagcctacgaccggcagctcgacagcggagacaacccgtacctcaagtacaaccacgccgacgccgagttccaggagcggctcaaagaagatacgtcttttgggggcaacctcgggcgagcagtcttccaggccaaaaagaggcttcttgaacctcttggtctggttgaggaagcggctaagacggctcctggaaagaagaggcctgtagagcactctcctgtggagccagactcctcctcgggaaccggaaaggcgggccagcagcctgcaagaaaaagattgaattttggtcagactggagacgcagactcagtcccagaccctcaaccaatcggagaacctcccgcagccccctcaggtgtgggatctcttacaatggctgcaggcggtggcgcaccaatggcagacaataacgagggcgccgacggagtgggtaattcctcgggaaattggcattgcgattccacatggatgggcgacagagtcatcaccaccagcacccgaacctgggccctgcccacctacaacaaccacctctacaagcaaatctccaacagcacatctggaggatcttcaaatgacaacgcctacttcggctacagcaccccctgggggtattttgactttaacagattccactgccacttttcaccacgtgactggcagcgactcatcaacaacaactggggattccggcccaagagactcagcttcaagctcttcaacatccaggtcaaggaggtcacgcagaatgaaggcaccaagaccatcgccaataacctcaccagcaccatccaggtgtttacggactcggagtaccagctgccgtacgttctcggctctgcccaccagggctgcctgcctccgttcccggcggacgtgttcatgattccccagtacggctacctaacactcaacaacggtagtcaggccgtgggacgctcctccttctactgcctggaatactttccttcgcagatgctgagaaccggcaacaacttccagtttacttacaccttcgaggacgtgcctttccacagcagctacgcccacagccagagcttggaccggctgatgaatcctctgattgaccagtacctgtactacttgtctcggactcaaacaacaggaggcacgacaaatacgcagactctgggcttcagccaaggtgggcctaatacaatggccaatcaggcaaagaactggctgccaggaccctgttaccgccagcagcgagtatcaaagacatctgcggataacaacaacagtgaatactcgtggactggagctaccaagtaccacctcaatggcagagactctctggtgaatccgggcccggccatggcaagccacaaggacgatgaagaaaagttttttcctcagagcggggttctcatctttgggaagcaaggctcagagaaaacaaatgtggacattgaaaaggtcatgattacagacgaagaggaaatcaggacaaccaatcccgtggctacggagcagtatggttctgtatctaccaacctccagagaggccagagaggcgaaccaaaagcacgtgcaccagcccaggcggccaccgcagatgtcaacacacaaggcgttcttccaggcatggtctggcaggacagagatgtgtaccttcaggggcccatctgggcaaagattccacacacggacggacattttcacccctctcccctcatgggtggattcggacttaaacaccctccgcctcagatcctgatcaagaacacgcctgtacctgcggatcctccgaccaccttcaaccagtcaaagctgaactctttcatcacccagtattctactggccaagtcagcgtggagatcgagtgggagctgcagaaggaaaacagcaagcgctggaaccccgagatccagtacacctccaactactacaaatctacaagtgtggactttgctgttaatacagaaggcgtgtactctgaaccccgccccattggcacccgttacctcacccgtaatctgtaa

SEQ ID NO: 7 - DNA, 7360 bp, synthetic construct
  source 1..7360: mol_type = other DNA
ccgccatgccggggttttacgagattgtgattaaggtccccagcgaccttgacgagcatctgcccggcatttctgacagctttgtgaactgggtggccgagaaggaatgggagttgccgccagattctgacatggatctgaatctgattgagcaggcacccctgaccgtggccgagaagctgcagcgcgactttctgacggaatggcgccgtgtgagtaaggccccggaggcccttttctttgtgcaatttgagaagggagagagctacttccacatgcacgtgctcgtggaaaccaccggggtgaaatccatggttttgggacgtttcctgagtcagattcgcgaaaaactgattcagagaatttaccgcgggatcgagccgactttgccaaactggttcgcggtcacaaagaccagaaatggcgccggaggcgggaacaaggtggtggatgagtgctacatccccaattacttgctccccaaaacccagcctgagctccagtgggcgtggactaatatggaacagtatttaagcgcctgtttgaatctcacggagcgtaaacggttggtggcgcagcatctgacgcacgtgtcgcagacgcaggagcagaacaaagagaatcagaatcccaattctgatgcgccggtgatcagatcaaaaacttcagccaggtacatggagctggtcgggtggctcgtggacaaggggattacctcggagaagcagtggatccaggaggaccaggcctcatacatctccttcaatgcggcctccaactcgcggtcccaaatcaaggctgccttggacaatgcgggaaagattatgagcctgactaaaaccgcccccgactacctggtgggccagcagcccgtggaggacatttccagcaatcggatttataaaattttggaactaaacgggtacgatccccaatatgcggcttccgtctttctgggatgggccacgaaaaagttcggcaagaggaacaccatctggctgtttgggcctgcaactaccgggaagaccaacatcgcggaggccatagcccacactgtgcccttctacgggtgcgtaaactggaccaatgagaactttcccttcaacgactgtgtcgacaagatggtgatctggtgggaggaggggaagatgaccgccaaggtcgtggagtcggccaaagccattctcggaggaagcaaggtgcgcgtggaccagaaatgcaagtcctcggcccagatagacccgactcccgtgatcgtcacctccaacaccaacatgtgcgccgtgattgacgggaactcaacgaccttcgaacaccagcagccgttgcaagaccggatgttcaaatttgaactcacccgccgtctggatcatgactttgggaaggtcaccaagcaggaagtcaaagactttttccggtgggcaaaggatcacgtggttgaggtggagcatgaattctacgtcaaaaagggtggagccaagaaaagacccgcccccagtgacgcagatataagtgagcccaaacgggtgcgcgagtcagttgcgcagccatcgacgtcagacgcggaagcttcgatcaactacgcagacaggtaccaaaacaaatgttctcgtcacgtgggcatgaatctgatgctgtttccctgcagacaatgcgagagaatgaatcagaattcaaatatctgcttcactcacggacagaaagactgtttagagtgctttcccgtgtcagaatctcaacccgtttctgtcgtcaaaaaggcgtatcagaaactgtgctacattcatcatatcatgggaaaggtgccagacgcttgcactgcctgcgatctggtcaatgtggatttggatgactgcatctttgaacaataaatgatttaaatcaggtatggctgccgatggttatcttccagattggctcgaggacactctctctgaaggaataagacagtggtggaagctcaaacctggcccaccaccaccaaagcccgcagagcggcataaggacgacagcaggggtcttgtgcttcctgggtacaagtacctcggacccttcaacggactcgacaagggagagccggtcaacgaggcagacgccgcggccctcgagcacgacaaagcctacgaccggcagctcgacagcggagacaacccgtacctcaagtacaaccacgccgacgccgagttccaggagcggctcaaagaagatacgtcttttgggggcaacctcgggcgagcagtcttccaggccaaaaagaggcttcttgaacctcttggtctggttgaggaagcggctaagacggctcctggaaagaagaggcctgtagagcactctcctgtggagccagactcctcctcgggaaccggaaaggcgggccagcagcctgcaagaaaaagattgaattttggtcagactggagacgcagactcagtcccagaccctcaaccaatcggagaacctcccgcagccccctcaggtgtgggatctcttacaatggctgcaggcggtggcgcaccaatggcagacaataacgagggcgccgacggagtgggtaattcctcgggaaattggcattgcgattccacatggatgggcgacagagtcatcaccaccagcacccgaacctgggccctgcccacctacaacaaccacctctacaagcaaatctccaacagcacatctggaggatcttcaaatgacaacgcctacttcggctacagcaccccctgggggtattttgactttaacagattccactgccacttttcaccacgtgactggcagcgactcatcaacaacaactggggattccggcccaagagactcagcttcaagctcttcaacatccaggtcaaggaggtcacgcagaatgaaggcaccaagaccatcgccaataacctcaccagcaccatccaggtgtttacggactcggagtaccagctgccgtacgttctcggctctgcccaccagggctgcctgcctccgttcccggcggacgtgttcatgattccccagtacggctacctaacactcaacaacggtagtcaggccgtgggacgctcctccttctactgcctggaatactttccttcgcagatgctgagaaccggcaacaacttccagtttacttacaccttcgaggacgtgcctttccacagcagctacgcccacagccagagcttggaccggctgatgaatcctctgattgaccagtacctgtactacttgtctcggactcaaacaacaggaggcacgacaaatacgcagactctgggcttcagccaaggtgggcctaatacaatggccaatcaggcaaagaactggctgccaggaccctgttaccgccagcagcgagtatcaaagacatctgcggataacaacaacagtgaatactcgtggactggagctaccaagtaccacctcaatggcagagactctctggtgaatccgggcccggccatggcaagccacaaggacgatgaagaaaagttttttcctcagagcggggttctcatctttgggaagcaaggctcagagaaaacaaatgtggacattgaaaaggtcatgattacagacgaagaggaaatcaggacaaccaatcccgtggctacggagcagtatggttctgtatctaccaacctccagagaggccagagaggcgaaccaaaagcacgtgcaccagcccaggcggccaccgcagatgtcaacacacaaggcgttcttccaggcatggtctggcaggacagagatgtgtaccttcaggggcccatctgggcaaagattccacacacggacggacattttcacccctctcccctcatgggtggattcggacttaaacaccctccgcctcagatcctgatcaagaacacgcctgtacctgcggatcctccgaccaccttcaaccagtcaaagctgaactctttcatcacccagtattctactggccaagtcagcgtggagatcgagtgggagctgcagaaggaaaacagcaagcgctggaaccccgagatccagtacacctccaactactacaaatctacaagtgtggactttgctgttaatacagaaggcgtgtactctgaaccccgccccattggcacccgttacctcacccgtaatctgtaattgcctgttaatcaataaaccggttgattcgtttcagttgaactttggtctctgcgaagggcgaattcgtttaaacctgcaggactagaggtcctgtattagaggtcacgtgagtgttttgcgacattttgcgacaccatgtggtcacgctgggtatttaagcccgagtgagcacgcagggtctccattttgaagcgggaggtttgaacgcgcagccgccaagccgaattctgcagatatccatcacactggcggccgctcgactagagcggccgccaccgcggtggagctccagcttttgttccctttagtgagggttaattgcgcgcttggcgtaatcatggtcatagctgtttcctgtgtgaaattgttatccgctcacaattccacacaacatacgagccggaagcataaagtgtaaagcctggggtgcctaatgagtgagctaactcacattaattgcgttgcgctcactgcccgctttccagtcgggaaacctgtcgtgccagctgcattaatgaatcggccaacgcgcggggagaggcggtttgcgtattgggcgctcttccgcttcctcgctcactgactcgctgcgctcggtcgttcggctgcggcgagcggtatcagctcactcaaaggcggtaatacggttatccacagaatcaggggataacgcaggaaagaacatgtgagcaaaaggccagcaaaaggccaggaaccgtaaaaaggccgcgttgctggcgtttttccataggctccgcccccctgacgagcatcacaaaaatcgacgctcaagtcagaggtggcgaaacccgacaggactataaagataccaggcgtttccccctggaagctccctcgtgcgctctcctgttccgaccctgccgcttaccggatacctgtccgcctttctcccttcgggaagcgtggcgctttctcatagctcacgctgtaggtatctcagttcggtgtaggtcgttcgctccaagctgggctgtgtgcacgaaccccccgttcagcccgaccgctgcgccttatccggtaactatcgtcttgagtccaacccggtaagacacgacttatcgccactggcagcagccactggtaacaggattagcagagcgaggtatgtaggcggtgctacagagttcttgaagtggtggcctaactacggctacactagaagaacagtatttggtatctgcgctctgctgaagccagttaccttcggaaaaagagttggtagctcttgatccggcaaacaaaccaccgctggtagcggtggtttttttgtttgcaagcagcagattacgcgcagaaaaaaaggatctcaagaagatcctttgatcttttctacggggtctgacgctcagtggaacgaaaactcacgttaagggattttggtcatgagattatcaaaaaggatcttcacctagatccttttaaattaaaaatgaagttttaaatcaatctaaagtatatatgagtaaacttggtctgacagttaccaatgcttaatcagtgaggcacctatctcagcgatctgtctatttcgttcatccatagttgcctgactccccgtcgtgtagataactacgatacgggagggcttaccatctggccccagtgctgcaatgataccgcgagacccacgctcaccggctccagatttatcagcaataaaccagccagccggaagggccgagcgcagaagtggtcctgcaactttatccgcctccatccagtctattaattgttgccgggaagctagagtaagtagttcgccagttaatagtttgcgcaacgttgttgccattgctacaggcatcgtggtgtcacgctcgtcgtttggtatggcttcattcagctccggttcccaacgatcaaggcgagttacatgatcccccatgttgtgcaaaaaagcggttagctccttcggtcctccgatcgttgtcagaagtaagttggccgcagtgttatcactcatggttatggcagcactgcataattctcttactgtcatgccatccgtaagatgcttttctgtgactggtgagtactcaaccaagtcattctgagaatagtgtatgcggcgaccgagttgctcttgcccggcgtcaatacgggataataccgcgccacatagcagaactttaaaagtgctcatcattggaaaacgttcttcggggcgaaaactctcaaggatcttaccgctgttgagatccagttcgatgtaacccactcgtgcacccaactgatcttcagcatcttttactttcaccagcgtttctgggtgagcaaaaacaggaaggcaaaatgccgcaaaaaagggaataagggcgacacggaaatgttgaatactcatactcttcctttttcaatattattgaagcatttatcagggttattgtctcatgagcggatacatatttgaatgtatttagaaaaataaacaaataggggttccgcgcacatttccccgaaaagtgccacctaaattgtaagcgttaatattttgttaaaattcgcgttaaatttttgttaaatcagctcattttttaaccaataggccgaaatcggcaaaatcccttataaatcaaaagaatagaccgagatagggttgagtgttgttccagtttggaacaagagtccactattaaagaacgtggactccaacgtcaaagggcgaaaaaccgtctatcagggcgatggcccactacgtgaaccatcaccctaatcaagttttttggggtcgaggtgccgtaaagcactaaatcggaaccctaaagggagcccccgatttagagcttgacggggaaagccggcgaacgtggcgagaaaggaagggaagaaagcgaaaggagcgggcgctagggcgctggcaagtgtagcggtcacgctgcgcgtaaccaccacacccgccgcgcttaatgcgccgctacagggcgcgtcccattcgccattcaggctgcgcaactgttgggaagggcgatcggtgcgggcctcttcgctattacgccagctggcgaaagggggatgtgctgcaaggcgattaagttgggtaacgccagggttttcccagtcacgacgttgtaaaacgacggccagtgagcgcgcgtaatacgactcactatagggcgaattgggtaccgggccccccctcgatcgaggtcgacggtatcgggggagctcgcagggtctccattttgaagcgggaggtttgaacgcgcag

SEQ ID NO: 8 - DNA, 5526 bp, synthetic construct
  source 1..5526: mol_type = other DNA
cttccgcttcctcgctcactgactcgctgcgctcggtcgttcggctgcggcgagcggtatcagctcactcaaaggcggtaatacggttatccacagaatcaggggataacgcaggaaagaacatgtgagcaaaaggccagcaaaaggccaggaaccgtaaaaaggccgcgttgctggcgtttttccataggctccgcccccctgacgagcatcacaaaaatcgacgctcaagtcagaggtggcgaaacccgacaggactataaagataccaggcgtttccccctggaagctccctcgtgcgctctcctgttccgaccctgccgcttaccggatacctgtccgcctttctcccttcgggaagcgtggcgctttctcatagctcacgctgtaggtatctcagttcggtgtaggtcgttcgctccaagctgggctgtgtgcacgaaccccccgttcagcccgaccgctgcgccttatccggtaactatcgtcttgagtccaacccggtaagacacgacttatcgccactggcagcagccactggtaacaggattagcagagcgaggtatgtaggcggtgctacagagttcttgaagtggtggcctaactacggctacactagaagaacagtatttggtatctgcgctctgctgaagccagttaccttcggaaaaagagttggtagctcttgatccggcaaacaaaccaccgctggtagcggtggtttttttgtttgcaagcagcagattacgcgcagaaaaaaaggatctcaagaagatcctttgatcttttctacggggtctgacgctcagtggaacgaaaactcacgttaagggattttggtcatgagattatcaaaaaggatcttcacctagatccttttaaattaaaaatgaagttttaaatcaatctaaagtatatatgagtaaacttggtctgacagttaccaatgcttaatcagtgaggcacctatctcagcgatctgtctatttcgttcatccatagttgcctgactccccgtcgtgtagataactacgatacgggagggcttaccatctggccccagtgctgcaatgataccgcgagacccacgctcaccggctccagatttatcagcaataaaccagccagccggaagggccgagcgcagaagtggtcctgcaactttatccgcctccatccagtctattaattgttgccgggaagctagagtaagtagttcgccagttaatagtttgcgcaacgttgttgccattgctacaggcatcgtggtgtcacgctcgtcgtttggtatggcttcattcagctccggttcccaacgatcaaggcgagttacatgatcccccatgttgtgcaaaaaagcggttagctccttcggtcctccgatcgttgtcagaagtaagttggccgcagtgttatcactcatggttatggcagcactgcataattctcttactgtcatgccatccgtaagatgcttttctgtgactggtgagtactcaaccaagtcattctgagaatagtgtatgcggcgaccgagttgctcttgcccggcgtcaatacgggataataccgcgccacatagcagaactttaaaagtgctcatcattggaaaacgttcttcggggcgaaaactctcaaggatcttaccgctgttgagatccagttcgatgtaacccactcgtgcacccaactgatcttcagcatcttttactttcaccagcgtttctgggtgagcaaaaacaggaaggcaaaatgccgcaaaaaagggaataagggcgacacggaaatgttgaatactcatactcttcctttttcaatattattgaagcatttatcagggttattgtctcatgagcggatacatatttgaatgtatttagaaaaataaacaaataggggttccgcgcacatttccccgaaaagtgccacctaaattgtaagcgttaatattttgttaaaattcgcgttaaatttttgttaaatcagctcattttttaaccaataggccgaaatcggcaaaatcccttataaatcaaaagaatagaccgagatagggttgagtgttgttccagtttggaacaagagtccactattaaagaacgtggactccaacgtcaaagggcgaaaaaccgtctatcagggcgatggcccactacgtgaaccatcaccctaatcaagttttttggggtcgaggtgccgtaaagcactaaatcggaaccctaaagggagcccccgatttagagcttgacggggaaagccggcgaacgtggcgagaaaggaagggaagaaagcgaaaggagcgggcgctagggcgctggcaagtgtagcggtcacgctgcgcgtaaccaccacacccgccgcgcttaatgcgccgctacagggcgcgtcccattcgccattcaggctgcgcaactgttgggaagggcgatcggtgcgggcctcttcgctattacgccagctgcgcgctcgctcgctcactgaggccgcccgggcaaagcccgggcgtcgggcgacctttggtcgcccggcctcagtgagcgagcgagcgcgcagagagggagtggccaactccatcactaggggttccttgtagttaatgattaacccgccatgctacttatctacgtagccatgctctaggaagagtaccattgacgtcaataatgacgtatgttcccatagtaacgccaatagggactttccattgacgtcaatgggtggagtatttacggtaaactgcccacttggcagtacatcaagtgtatcatatgccaagtacgccccctattgacgtcaatgacggtaaatggcccgcctggcattatgcccagtacatgaccttatgggactttcctacttggcagtacatctacgtattagtcatcgctattaccatggtcgaggtgagccccacgttctgcttcactctccccatctcccccccctccccacccccaattttgtatttatttattttttaattattttgtgcagcgatgggggcggggggggggggggggcgcgcgccgggcggggcggggcggggcgaggggcggggcggggcgaggcggagaggtgcggcggcagccaatcagagcggcgcgctccgaaagtttccttttatggcgaggcggcggcggcggcggccctataaaaagcgaagcgcgcggcgggcgggagtcgctgcgcgctgccttcgccccgtgccccgctccgccgccgcctcgcgccgcccgccccggctctgactgaccgcgttactcccacaggtgagcgggcgggacggcccttctcctccgggctgtaattagcgcttggtttaatgacggcttgtttcttttctgtggctgcgtgaaagccttgaggggctccgggagggccctttgtgcggggggagcggctcggggctgtccgcggggggacggctgccttcgggggggacggggcagggcggggttcggcttctggcgtgtgaccggcggctctagagcctctgctaaccatgttcatgccttcttctttttcctacagctcctgggcaacgtgctggttattgtgctgtctcatcattttggcaaagaattggatccgccaccatggtgagcaagggcgaggagctgttcaccggggtggtgcccatcctggtcgagctggacggcgacgtaaacggccacaagttcagcgtgtccggcgagggcgagggcgatgccacctacggcaagctgaccctgaagttcatttgcaccaccggcaagctgcccgtgccctggcccaccctcgtgaccaccctgacctacggcgtgcagtgcttcagccgctaccccgaccacatgaagcagcacgacttcttcaagtccgccatgcccgaaggctacgtccaggagcgcaccatcttcttcaaggacgacggcaactacaagacccgcgccgaggtgaagttcgagggcgacaccctggtgaaccgcatcgagctgaagggcatcgacttcaaggaggacggcaacatcctggggcacaagctggagtacaactacaacagccacaacgtctatatcatggccgacaagcagaagaacggcatcaaggtgaacttcaagatccgccacaacatcgaggacggcagcgtgcagctcgccgaccactaccagcagaacacccccatcggcgacggccccgtgctgctgcccgacaaccactacctgagcacccagtccgccctgagcaaagaccccaacgagaagcgcgatcacatggtcctgctggagttcgtgaccgccgccgggatcactctcggcatggacgagctgtacaagtccggactcagatctgatccaaaaaagaagagaaaggtagatccaaaaaagaagagaaaggtagatccaaaaaagaagagaaaggtataagaattcgatatcaagcttatcgataatcaacctctggattacaaaatttgtgaaagattgactggtattcttaactatgttgctccttttacgctatgtggatacgctgctttaatgcctttgtatcatgctattgcttcccgtatggctttcattttctcctccttgtataaatcctggttgctgtctctttatgaggagttgtggcccgttgtcaggcaacgtggcgtggtgtgcactgtgtttgctgacgcaacccccactggttggggcattgccaccacctgtcagctcctttccgggactttcgctttccccctccctattgccacggcggaactcatcgccgcctgccttgcccgctgctggacaggggctcggctgttgggcactgacaattccgtggtgttgtcggggaaatcatcgtcctttccttggctgctcgcctgtgttgccacctggattctgcgcgggacgtccttctgctacgtcccttcggccctcaatccagcggaccttccttcccgcggcctgctgccggctctgcggcctcttccgcgtcttcgccttcgccctcagacgagtcggatctccctttgggccgcctccccgcatcgataccgtcgacccgggcggccgcttcgagcagacatgataagatacattgatgagtttggacaaaccacaactagaatgcagtgaaaaaaatgctttatttgtgaaatttgtgatgctattgctttatttgtaaccattataagctgcaataaacaagttaacaacaacaattgcattcattttatgtttcaggttcagggggagatgtgggaggttttttaaagcaagtaaaacctctacaaatgtggtaaaatcgataaggatcttcctagagcatggctacgtagataagtagcatggcgggttaatcattaactacaaggaacccctagtgatggagttggccactccctctctgcgcgctcgctcgctcactgaggccgggcgaccaaaggtcgcccgacgcccgggctttgcccgggcggcctcagtgagcgagcgagcgcgcagctgcattaatgaatcggccaacgcgcggggagaggcggtttgcgtattgggcgct

SEQ ID NO: 9 - DNA, 5547 bp, synthetic construct
  source 1..5547: mol_type = other DNA
cttccgcttcctcgctcactgactcgctgcgctcggtcgttcggctgcggcgagcggtatcagctcactcaaaggcggtaatacggttatccacagaatcaggggataacgcaggaaagaacatgtgagcaaaaggccagcaaaaggccaggaaccgtaaaaaggccgcgttgctggcgtttttccataggctccgcccccctgacgagcatcacaaaaatcgacgctcaagtcagaggtggcgaaacccgacaggactataaagataccaggcgtttccccctggaagctccctcgtgcgctctcctgttccgaccctgccgcttaccggatacctgtccgcctttctcccttcgggaagcgtggcgctttctcatagctcacgctgtaggtatctcagttcggtgtaggtcgttcgctccaagctgggctgtgtgcacgaaccccccgttcagcccgaccgctgcgccttatccggtaactatcgtcttgagtccaacccggtaagacacgacttatcgccactggcagcagccactggtaacaggattagcagagcgaggtatgtaggcggtgctacagagttcttgaagtggtggcctaactacggctacactagaagaacagtatttggtatctgcgctctgctgaagccagttaccttcggaaaaagagttggtagctcttgatccggcaaacaaaccaccgctggtagcggtggtttttttgtttgcaagcagcagattacgcgcagaaaaaaaggatctcaagaagatcctttgatcttttctacggggtctgacgctcagtggaacgaaaactcacgttaagggattttggtcatgagattatcaaaaaggatcttcacctagatccttttaaattaaaaatgaagttttaaatcaatctaaagtatatatgagtaaacttggtctgacagttaccaatgcttaatcagtgaggcacctatctcagcgatctgtctatttcgttcatccatagttgcctgactccccgtcgtgtagataactacgatacgggagggcttaccatctggccccagtgctgcaatgataccgcgagacccacgctcaccggctccagatttatcagcaataaaccagccagccggaagggccgagcgcagaagtggtcctgcaactttatccgcctccatccagtctattaattgttgccgggaagctagagtaagtagttcgccagttaatagtttgcgcaacgttgttgccattgctacaggcatcgtggtgtcacgctcgtcgtttggtatggcttcattcagctccggttcccaacgatcaaggcgagttacatgatcccccatgttgtgcaaaaaagcggttagctccttcggtcctccgatcgttgtcagaagtaagttggccgcagtgttatcactcatggttatggcagcactgcataattctcttactgtcatgccatccgtaagatgcttttctgtgactggtgagtactcaaccaagtcattctgagaatagtgtatgcggcgaccgagttgctcttgcccggcgtcaatacgggataataccgcgccacatagcagaactttaaaagtgctcatcattggaaaacgttcttcggggcgaaaactctcaaggatcttaccgctgttgagatccagttcgatgtaacccactcgtgcacccaactgatcttcagcatcttttactttcaccagcgtttctgggtgagcaaaaacaggaaggcaaaatgccgcaaaaaagggaataagggcgacacggaaatgttgaatactcatactcttcctttttcaatattattgaagcatttatcagggttattgtctcatgagcggatacatatttgaatgtatttagaaaaataaacaaataggggttccgcgcacatttccccgaaaagtgccacctaaattgtaagcgttaatattttgttaaaattcgcgttaaatttttgttaaatcagctcattttttaaccaataggccgaaatcggcaaaatcccttataaatcaaaagaatagaccgagatagggttgagtgttgttccagtttggaacaagagtccactattaaagaacgtggactccaacgtcaaagggcgaaaaaccgtctatcagggcgatggcccactacgtgaaccatcaccctaatcaagttttttggggtcgaggtgccgtaaagcactaaatcggaaccctaaagggagcccccgatttagagcttgacggggaaagccggcgaacgtggcgagaaaggaagggaagaaagcgaaaggagcgggcgctagggcgctggcaagtgtagcggtcacgctgcgcgtaaccaccacacccgccgcgcttaatgcgccgctacagggcgcgtcccattcgccattcaggctgcgcaactgttgggaagggcgatcggtgcgggcctcttcgctattacgccagctgcgcgctcgctcgctcactgaggccgcccgggcaaagcccgggcgtcgggcgacctttggtcgcccggcctcagtgagcgagcgagcgcgcagagagggagtggccaactccatcactaggggttccttgtagttaatgattaacccgccatgctacttatctacgtagccatgctctaggaagagtaccattgacgtcaataatgacgtatgttcccatagtaacgccaatagggactttccattgacgtcaatgggtggagtatttacggtaaactgcccacttggcagtacatcaagtgtatcatatgccaagtacgccccctattgacgtcaatgacggtaaatggcccgcctggcattatgcccagtacatgaccttatgggactttcctacttggcagtacatctacgtattagtcatcgctattaccatggtcgaggtgagccccacgttctgcttcactctccccatctcccccccctccccacccccaattttgtatttatttattttttaattattttgtgcagcgatgggggcggggggggggggggggcgcgcgccgggcggggcggggcggggcgaggggcggggcggggcgaggcggagaggtgcggcggcagccaatcagagcggcgcgctccgaaagtttccttttatggcgaggcggcggcggcggcggccctataaaaagcgaagcgcgcggcgggcgggagtcgctgcgcgctgccttcgccccgtgccccgctccgccgccgcctcgcgccgcccgccccggctctgactgaccgcgttactcccacaggtgagcgggcgggacggcccttctcctccgggctgtaattagcgcttggtttaatgacggcttgtttcttttctgtggctgcgtgaaagccttgaggggctccgggagggccctttgtgcggggggagcggctcggggctgtccgcggggggacggctgccttcgggggggacggggcagggcggggttcggcttctggcgtgtgaccggcggctctagagcctctgctaaccatgttcatgccttcttctttttcctacagctcctgggcaacgtgctggttattgtgctgtctcatcattttggcaaagaattggatccgccaccatggcatatccgtatgatgtgccggattatgcggtgagcaagggcgaggaggataacatggccatcatcaaggagttcatgcgcttcaaggtgcacatggagggctccgtgaacggccacgagttcgagatcgagggcgagggcgagggccgcccctacgagggcacccagaccgccaagctgaaggtgaccaagggtggccccctgcccttcgcctgggacatcctgtcccctcagttcatgtacggctccaaggcctacgtgaagcaccccgccgacatccccgactacttgaagctgtccttccccgagggcttcaagtgggagcgcgtgatgaacttcgaggacggcggcgtggtgaccgtgacccaggactcctccctgcaggacggcgagttcatctacaaggtgaagctgcgcggcaccaacttcccctccgacggccccgtaatgcagaagaagaccatgggctgggaggcctcctccgagcggatgtaccccgaggacggcgccctgaagggcgagatcaagcagaggctgaagctgaaggacggcggccactacgacgctgaggtcaagaccacctacaaggccaagaagcccgtgcagctgcccggcgcctacaacgtcaacatcaagttggacatcacctcccacaacgaggactacaccatcgtggaacagtacgaacgcgccgagggccgccactccaccggcggcatggacgagctgtacaagtccggactcagatctgatccaaaaaagaagagaaaggtagatccaaaaaagaagagaaaggtagatccaaaaaagaagagaaaggtataagaattcgatatcaagcttatcgataatcaacctctggattacaaaatttgtgaaagattgactggtattcttaactatgttgctccttttacgctatgtggatacgctgctttaatgcctttgtatcatgctattgcttcccgtatggctttcattttctcctccttgtataaatcctggttgctgtctctttatgaggagttgtggcccgttgtcaggcaacgtggcgtggtgtgcactgtgtttgctgacgcaacccccactggttggggcattgccaccacctgtcagctcctttccgggactttcgctttccccctccctattgccacggcggaactcatcgccgcctgccttgcccgctgctggacaggggctcggctgttgggcactgacaattccgtggtgttgtcggggaaatcatcgtcctttccttggctgctcgcctgtgttgccacctggattctgcgcgggacgtccttctgctacgtcccttcggccctcaatccagcggaccttccttcccgcggcctgctgccggctctgcggcctcttccgcgtcttcgccttcgccctcagacgagtcggatctccctttgggccgcctccccgcatcgataccgtcgacccgggcggccgcttcgagcagacatgataagatacattgatgagtttggacaaaccacaactagaatgcagtgaaaaaaatgctttatttgtgaaatttgtgatgctattgctttatttgtaaccattataagctgcaataaacaagttaacaacaacaattgcattcattttatgtttcaggttcagggggagatgtgggaggttttttaaagcaagtaaaacctctacaaatgtggtaaaatcgataaggatcttcctagagcatggctacgtagataagtagcatggcgggttaatcattaactacaaggaacccctagtgatggagttggccactccctctctgcgcgctcgctcgctcactgaggccgggcgaccaaaggtcgcccgacgcccgggctttgcccgggcggcctcagtgagcgagcgagcgcgcagctgcattaatgaatcggccaacgcgcggggagaggcggtttgcgtattgggcgct

SEQ ID NO: 10 - protein, 14 aa, synthetic construct
NAAAPRGDLAPAAR

SEQ ID NO: 11 - protein, 14 aa, synthetic construct
NAAARGDTATLAAR

SEQ ID NO: 12 - protein, 14 aa, synthetic construct
NAAARGDQQSLAAR

SEQ ID NO: 13 - protein, 14 aa, synthetic construct
NAAAPRGDLRPAAR

SEQ ID NO: 14 - protein, 749 aa, synthetic construct
MAADGYLPDWLEDTLSEGIRQWWKLKPGPPPPKPAERHKDDSRGLVLPGYKYLGPFNGLDKGEPVNEADAAALEHDKAYDRQLDSGDNPYLKYNHADAEFQERLKEDTSFGGNLGRAVFQAKKRLLEPLGLVEEAAKTAPGKKRPVEHSPVEPDSSSGTGKAGQQPARKRLNFGQTGDADSVPDPQPIGEPPAAPSGVGSLTMAAGGGAPMADNNEGADGVGNSSGNWHCDSTWMGDRVITTSTRTWALPTYNNHLYKQISNSTSGGSSNDNAYFGYSTPWGYFDFNRFHCHFSPRDWQRLINNNWGFRPKRLSFKLFNIQVKEVTQNEGTKTIANNLTSTIQVFTDSEYQLPYVLGSAHQGCLPPFPADVFMIPQYGYLTLNNGSQAVGRSSFYCLEYFPSQMLRTGNNFQFTYTFEDVPFHSSYAHSQSLDRLMNPLIDQYLYYLSRTQTTGGTTNTQTLGFSQGGPNTMANQAKNWLPGPCYRQQRVSKTSADNNNSEYSWTGATKYHLNGRDSLVNPGPAMASHKDDEEKFFPQSGVLIFGKQGSEKTNVDIEKVMITDEEEIRTTNPVATEQYGSVSTNLQRGNAAAPRGDLAPAARQAATADVNTQGVLPGMVWQDRDVYLQGPIWAKIPHTDGHFHPSPLMGGFGLKHPPPQILIKNTPVPADPPTTFNQSKLNSFITQYSTGQVSVEIEWELQKENSKRWNPEIQYTSNYYKSTSVDFAVNTEGVYSEPRPIGTRYLTRNL

SEQ ID NO: 15 - protein, 749 aa, synthetic construct
MAADGYLPDWLEDTLSEGIRQWWKLKPGPPPPKPAERHKDDSRGLVLPGYKYLGPFNGLDKGEPVNEADAAALEHDKAYDRQLDSGDNPYLKYNHADAEFQERLKEDTSFGGNLGRAVFQAKKRLLEPLGLVEEAAKTAPGKKRPVEHSPVEPDSSSGTGKAGQQPARKRLNFGQTGDADSVPDPQPIGEPPAAPSGVGSLTMAAGGGAPMADNNEGADGVGNSSGNWHCDSTWMGDRVITTSTRTWALPTYNNHLYKQISNSTSGGSSNDNAYFGYSTPWGYFDFNRFHCHFSPRDWQRLINNNWGFRPKRLSFKLFNIQVKEVTQNEGTKTIANNLTSTIQVFTDSEYQLPYVLGSAHQGCLPPFPADVFMIPQYGYLTLNNGSQAVGRSSFYCLEYFPSQMLRTGNNFQFTYTFEDVPFHSSYAHSQSLDRLMNPLIDQYLYYLSRTQTTGGTTNTQTLGFSQGGPNTMANQAKNWLPGPCYRQQRVSKTSADNNNSEYSWTGATKYHLNGRDSLVNPGPAMASHKDDEEKFFPQSGVLIFGKQGSEKTNVDIEKVMITDEEEIRTTNPVATEQYGSVSTNLQRGNAAARGDTATLAARQAATADVNTQGVLPGMVWQDRDVYLQGPIWAKIPHTDGHFHPSPLMGGFGLKHPPPQILIKNTPVPADPPTTFNQSKLNSFITQYSTGQVSVEIEWELQKENSKRWNPEIQYTSNYYKSTSVDFAVNTEGVYSEPRPIGTRYLTRNL

SEQ ID NO: 16 - protein, 749 aa, synthetic construct
MAADGYLPDWLEDTLSEGIRQWWKLKPGPPPPKPAERHKDDSRGLVLPGYKYLGPFNGLDKGEPVNEADAAALEHDKAYDRQLDSGDNPYLKYNHADAEFQERLKEDTSFGGNLGRAVFQAKKRLLEPLGLVEEAAKTAPGKKRPVEHSPVEPDSSSGTGKAGQQPARKRLNFGQTGDADSVPDPQPIGEPPAAPSGVGSLTMAAGGGAPMADNNEGADGVGNSSGNWHCDSTWMGDRVITTSTRTWALPTYNNHLYKQISNSTSGGSSNDNAYFGYSTPWGYFDFNRFHCHFSPRDWQRLINNNWGFRPKRLSFKLFNIQVKEVTQNEGTKTIANNLTSTIQVFTDSEYQLPYVLGSAHQGCLPPFPADVFMIPQYGYLTLNNGSQAVGRSSFYCLEYFPSQMLRTGNNFQFTYTFEDVPFHSSYAHSQSLDRLMNPLIDQYLYYLSRTQTTGGTTNTQTLGFSQGGPNTMANQAKNWLPGPCYRQQRVSKTSADNNNSEYSWTGATKYHLNGRDSLVNPGPAMASHKDDEEKFFPQSGVLIFGKQGSEKTNVDIEKVMITDEEEIRTTNPVATEQYGSVSTNLQRGNAAARGDQQSLAARQAATADVNTQGVLPGMVWQDRDVYLQGPIWAKIPHTDGHFHPSPLMGGFGLKHPPPQILIKNTPVPADPPTTFNQSKLNSFITQYSTGQVSVEIEWELQKENSKRWNPEIQYTSNYYKSTSVDFAVNTEGVYSEPRPIGTRYLTRNL

SEQ ID NO: 17 - protein, 749 aa, synthetic construct
MAADGYLPDWLEDTLSEGIRQWWKLKPGPPPPKPAERHKDDSRGLVLPGYKYLGPFNGLDKGEPVNEADAAALEHDKAYDRQLDSGDNPYLKYNHADAEFQERLKEDTSFGGNLGRAVFQAKKRLLEPLGLVEEAAKTAPGKKRPVEHSPVEPDSSSGTGKAGQQPARKRLNFGQTGDADSVPDPQPIGEPPAAPSGVGSLTMAAGGGAPMADNNEGADGVGNSSGNWHCDSTWMGDRVITTSTRTWALPTYNNHLYKQISNSTSGGSSNDNAYFGYSTPWGYFDFNRFHCHFSPRDWQRLINNNWGFRPKRLSFKLFNIQVKEVTQNEGTKTIANNLTSTIQVFTDSEYQLPYVLGSAHQGCLPPFPADVFMIPQYGYLTLNNGSQAVGRSSFYCLEYFPSQMLRTGNNFQFTYTFEDVPFHSSYAHSQSLDRLMNPLIDQYLYYLSRTQTTGGTTNTQTLGFSQGGPNTMANQAKNWLPGPCYRQQRVSKTSADNNNSEYSWTGATKYHLNGRDSLVNPGPAMASHKDDEEKFFPQSGVLIFGKQGSEKTNVDIEKVMITDEEEIRTTNPVATEQYGSVSTNLQRGNAAAPRGDLRPAARQAATADVNTQGVLPGMVWQDRDVYLQGPIWAKIPHTDGHFHPSPLMGGFGLKHPPPQILIKNTPVPADPPTTFNQSKLNSFITQYSTGQVSVEIEWELQKENSKRWNPEIQYTSNYYKSTSVDFAVNTEGVYSEPRPIGTRYLTRNL

SEQ ID NO: 18 - DNA, 2250 bp, synthetic construct
  source 1..2250: mol_type = other DNA
atggctgccgatggttatcttccagattggctcgaggacactctctctgaaggaataagacagtggtggaagctcaaacctggcccaccaccaccaaagcccgcagagcggcataaggacgacagcaggggtcttgtgcttcctgggtacaagtacctcggacccttcaacggactcgacaagggagagccggtcaacgaggcagacgccgcggccctcgagcacgacaaagcctacgaccggcagctcgacagcggagacaacccgtacctcaagtacaaccacgccgacgccgagttccaggagcggctcaaagaagatacgtcttttgggggcaacctcgggcgagcagtcttccaggccaaaaagaggcttcttgaacctcttggtctggttgaggaagcggctaagacggctcctggaaagaagaggcctgtagagcactctcctgtggagccagactcctcctcgggaaccggaaaggcgggccagcagcctgcaagaaaaagattgaattttggtcagactggagacgcagactcagtcccagaccctcaaccaatcggagaacctcccgcagccccctcaggtgtgggatctcttacaatggctgcaggcggtggcgcaccaatggcagacaataacgagggcgccgacggagtgggtaattcctcgggaaattggcattgcgattccacatggatgggcgacagagtcatcaccaccagcacccgaacctgggccctgcccacctacaacaaccacctctacaagcaaatctccaacagcacatctggaggatcttcaaatgacaacgcctacttcggctacagcaccccctgggggtattttgactttaacagattccactgccacttttcaccacgtgactggcagcgactcatcaacaacaactggggattccggcccaagagactcagcttcaagctcttcaacatccaggtcaaggaggtcacgcagaatgaaggcaccaagaccatcgccaataacctcaccagcaccatccaggtgtttacggactcggagtaccagctgccgtacgttctcggctctgcccaccagggctgcctgcctccgttcccggcggacgtgttcatgattccccagtacggctacctaacactcaacaacggtagtcaggccgtgggacgctcctccttctactgcctggaatactttccttcgcagatgctgagaaccggcaacaacttccagtttacttacaccttcgaggacgtgcctttccacagcagctacgcccacagccagagcttggaccggctgatgaatcctctgattgaccagtacctgtactacttgtctcggactcaaacaacaggaggcacgacaaatacgcagactctgggcttcagccaaggtgggcctaatacaatggccaatcaggcaaagaactggctgccaggaccctgttaccgccagcagcgagtatcaaagacatctgcggataacaacaacagtgaatactcgtggactggagctaccaagtaccacctcaatggcagagactctctggtgaatccgggcccggccatggcaagccacaaggacgatgaagaaaagttttttcctcagagcggggttctcatctttgggaagcaaggctcagagaaaacaaatgtggacattgaaaaggtcatgattacagacgaagaggaaatcaggacaaccaatcccgtggctacggagcagtatggttctgtatctaccaacctccagagaggcaacgcagcagcaccacgtggtgatctggcaccagcagcaagacaagcagctaccgcagatgtcaacacacaaggcgttcttccaggcatggtctggcaggacagagatgtgtaccttcaggggcccatctgggcaaagattccacacacggacggacattttcacccctctcccctcatgggtggattcggacttaaacaccctccgcctcagatcctgatcaagaacacgcctgtacctgcggatcctccgaccaccttcaaccagtcaaagctgaactctttcatcacccagtattctactggccaagtcagcgtggagatcgagtgggagctgcagaaggaaaacagcaagcgctggaaccccgagatccagtacacctccaactactacaaatctacaagtgtggactttgctgttaatacagaaggcgtgtactctgaaccccgccccattggcacccgttacctcacccgtaatctgtaa

SEQ ID NO: 19 - DNA, 2250 bp, synthetic construct
  source 1..2250: mol_type = other DNA
atggctgccgatggttatcttccagattggctcgaggacactctctctgaaggaataagacagtggtggaagctcaaacctggcccaccaccaccaaagcccgcagagcggcataaggacgacagcaggggtcttgtgcttcctgggtacaagtacctcggacccttcaacggactcgacaagggagagccggtcaacgaggcagacgccgcggccctcgagcacgacaaagcctacgaccggcagctcgacagcggagacaacccgtacctcaagtacaaccacgccgacgccgagttccaggagcggctcaaagaagatacgtcttttgggggcaacctcgggcgagcagtcttccaggccaaaaagaggcttcttgaacctcttggtctggttgaggaagcggctaagacggctcctggaaagaagaggcctgtagagcactctcctgtggagccagactcctcctcgggaaccggaaaggcgggccagcagcctgcaagaaaaagattgaattttggtcagactggagacgcagactcagtcccagaccctcaaccaatcggagaacctcccgcagccccctcaggtgtgggatctcttacaatggctgcaggcggtggcgcaccaatggcagacaataacgagggcgccgacggagtgggtaattcctcgggaaattggcattgcgattccacatggatgggcgacagagtcatcaccaccagcacccgaacctgggccctgcccacctacaacaaccacctctacaagcaaatctccaacagcacatctggaggatcttcaaatgacaacgcctacttcggctacagcaccccctgggggtattttgactttaacagattccactgccacttttcaccacgtgactggcagcgactcatcaacaacaactggggattccggcccaagagactcagcttcaagctcttcaacatccaggtcaaggaggtcacgcagaatgaaggcaccaagaccatcgccaataacctcaccagcaccatccaggtgtttacggactcggagtaccagctgccgtacgttctcggctctgcccaccagggctgcctgcctccgttcccggcggacgtgttcatgattccccagtacggctacctaacactcaacaacggtagtcaggccgtgggacgctcctccttctactgcctggaatactttccttcgcagatgctgagaaccggcaacaacttccagtttacttacaccttcgaggacgtgcctttccacagcagctacgcccacagccagagcttggaccggctgatgaatcctctgattgaccagtacctgtactacttgtctcggactcaaacaacaggaggcacgacaaatacgcagactctgggcttcagccaaggtgggcctaatacaatggccaatcaggcaaagaactggctgccaggaccctgttaccgccagcagcgagtatcaaagacatctgcggataacaacaacagtgaatactcgtggactggagctaccaagtaccacctcaatggcagagactctctggtgaatccgggcccggccatggcaagccacaaggacgatgaagaaaagttttttcctcagagcggggttctcatctttgggaagcaaggctcagagaaaacaaatgtggacattgaaaaggtcatgattacagacgaagaggaaatcaggacaaccaatcccgtggctacggagcagtatggttctgtatctaccaacctccagagaggcaacgcagcagcacgtggtgatactgcaactctggcagcaagacaagcagctaccgcagatgtcaacacacaaggcgttcttccaggcatggtctggcaggacagagatgtgtaccttcaggggcccatctgggcaaagattccacacacggacggacattttcacccctctcccctcatgggtggattcggacttaaacaccctccgcctcagatcctgatcaagaacacgcctgtacctgcggatcctccgaccaccttcaaccagtcaaagctgaactctttcatcacccagtattctactggccaagtcagcgtggagatcgagtgggagctgcagaaggaaaacagcaagcgctggaaccccgagatccagtacacctccaactactacaaatctacaagtgtggactttgctgttaatacagaaggcgtgtactctgaaccccgccccattggcacccgttacctcacccgtaatctgtaa

SEQ ID NO: 20 - DNA, 2250 bp, synthetic construct
  source 1..2250: mol_type = other DNA
atggctgccgatggttatcttccagattggctcgaggacactctctctgaaggaataagacagtggtggaagctcaaacctggcccaccaccaccaaagcccgcagagcggcataaggacgacagcaggggtcttgtgcttcctgggtacaagtacctcggacccttcaacggactcgacaagggagagccggtcaacgaggcagacgccgcggccctcgagcacgacaaagcctacgaccggcagctcgacagcggagacaacccgtacctcaagtacaaccacgccgacgccgagttccaggagcggctcaaagaagatacgtcttttgggggcaacctcgggcgagcagtcttccaggccaaaaagaggcttcttgaacctcttggtctggttgaggaagcggctaagacggctcctggaaagaagaggcctgtagagcactctcctgtggagccagactcctcctcgggaaccggaaaggcgggccagcagcctgcaagaaaaagattgaattttggtcagactggagacgcagactcagtcccagaccctcaaccaatcggagaacctcccgcagccccctcaggtgtgggatctcttacaatggctgcaggcggtggcgcaccaatggcagacaataacgagggcgccgacggagtgggtaattcctcgggaaattggcattgcgattccacatggatgggcgacagagtcatcaccaccagcacccgaacctgggccctgcccacctacaacaaccacctctacaagcaaatctccaacagcacatctggaggatcttcaaatgacaacgcctacttcggctacagcaccccctgggggtattttgactttaacagattccactgccacttttcaccacgtgactggcagcgactcatcaacaacaactggggattccggcccaagagactcagcttcaagctcttcaacatccaggtcaaggaggtcacgcagaatgaaggcaccaagaccatcgccaataacctcaccagcaccatccaggtgtttacggactcggagtaccagctgccgtacgttctcggctctgcccaccagggctgcctgcctccgttcccggcggacgtgttcatgattccccagtacggctacctaacactcaacaacggtagtcaggccgtgggacgctcctccttctactgcctggaatactttccttcgcagatgctgagaaccggcaacaacttccagtttacttacaccttcgaggacgtgcctttccacagcagctacgcccacagccagagcttggaccggctgatgaatcctctgattgaccagtacctgtactacttgtctcggactcaaacaacaggaggcacgacaaatacgcagactctgggcttcagccaaggtgggcctaatacaatggccaatcaggcaaagaactggctgccaggaccctgttaccgccagcagcgagtatcaaagacatctgcggataacaacaacagtgaatactcgtggactggagctaccaagtaccacctcaatggcagagactctctggtgaatccgggcccggccatggcaagccacaaggacgatgaagaaaagttttttcctcagagcggggttctcatctttgggaagcaaggctcagagaaaacaaatgtggacattgaaaaggtcatgattacagacgaagaggaaatcaggacaaccaatcccgtggctacggagcagtatggttctgtatctaccaacctccagagaggcaacgcagcagcacgtggtgatcagcagtctctggcagcaagacaagcagctaccgcagatgtcaacacacaaggcgttcttccaggcatggtctggcaggacagagatgtgtaccttcaggggcccatctgggcaaagattccacacacggacggacattttcacccctctcccctcatgggtggattcggacttaaacaccctccgcctcagatcctgatcaagaacacgcctgtacctgcggatcctccgaccaccttcaaccagtcaaagctgaactctttcatcacccagtattctactggccaagtcagcgtggagatcgagtgggagctgcagaaggaaaacagcaagcgctggaaccccgagatccagtacacctccaactactacaaatctacaagtgtggactttgctgttaatacagaaggcgtgtactctgaaccccgccccattggcacccgttacctcacccgtaatctgtaa

SEQ ID NO: 21 - DNA, 2250 bp, synthetic construct
  source 1..2250: mol_type = other DNA
atggctgccgatggttatcttccagattggctcgaggacactctctctgaaggaataagacagtggtggaagctcaaacctggcccaccaccaccaaagcccgcagagcggcataaggacgacagcaggggtcttgtgcttcctgggtacaagtacctcggacccttcaacggactcgacaagggagagccggtcaacgaggcagacgccgcggccctcgagcacgacaaagcctacgaccggcagctcgacagcggagacaacccgtacctcaagtacaaccacgccgacgccgagttccaggagcggctcaaagaagatacgtcttttgggggcaacctcgggcgagcagtcttccaggccaaaaagaggcttcttgaacctcttggtctggttgaggaagcggctaagacggctcctggaaagaagaggcctgtagagcactctcctgtggagccagactcctcctcgggaaccggaaaggcgggccagcagcctgcaagaaaaagattgaattttggtcagactggagacgcagactcagtcccagaccctcaaccaatcggagaacctcccgcagccccctcaggtgtgggatctcttacaatggctgcaggcggtggcgcaccaatggcagacaataacgagggcgccgacggagtgggtaattcctcgggaaattggcattgcgattccacatggatgggcgacagagtcatcaccaccagcacccgaacctgggccctgcccacctacaacaaccacctctacaagcaaatctccaacagcacatctggaggatcttcaaatgacaacgcctacttcggctacagcaccccctgggggtattttgactttaacagattccactgccacttttcaccacgtgactggcagcgactcatcaacaacaactggggattccggcccaagagactcagcttcaagctcttcaacatccaggtcaaggaggtcacgcagaatgaaggcaccaagaccatcgccaataacctcaccagcaccatccaggtgtttacggactcggagtaccagctgccgtacgttctcggctctgcccaccagggctgcctgcctccgttcccggcggacgtgttcatgattccccagtacggctacctaacactcaacaacggtagtcaggccgtgggacgctcctccttctactgcctggaatactttccttcgcagatgctgagaaccggcaacaacttccagtttacttacaccttcgaggacgtgcctttccacagcagctacgcccacagccagagcttggaccggctgatgaatcctctgattgaccagtacctgtactacttgtctcggactcaaacaacaggaggcacgacaaatacgcagactctgggcttcagccaaggtgggcctaatacaatggccaatcaggcaaagaactggctgccaggaccctgttaccgccagcagcgagtatcaaagacatctgcggataacaacaacagtgaatactcgtggactggagctaccaagtaccacctcaatggcagagactctctggtgaatccgggcccggccatggcaagccacaaggacgatgaagaaaagttttttcctcagagcggggttctcatctttgggaagcaaggctcagagaaaacaaatgtggacattgaaaaggtcatgattacagacgaagaggaaatcaggacaaccaatcccgtggctacggagcagtatggttctgtatctaccaacctccagagaggcaacgcagcagcaccacgtggtgatctgcgtccagcagcaagacaagcagctaccgcagatgtcaacacacaaggcgttcttccaggcatggtctggcaggacagagatgtgtaccttcaggggcccatctgggcaaagattccacacacggacggacattttcacccctctcccctcatgggtggattcggacttaaacaccctccgcctcagatcctgatcaagaacacgcctgtacctgcggatcctccgaccaccttcaaccagtcaaagctgaactctttcatcacccagtattctactggccaagtcagcgtggagatcgagtgggagctgcagaaggaaaacagcaagcgctggaaccccgagatccagtacacctccaactactacaaatctacaagtgtggactttgctgttaatacagaaggcgtgtactctgaaccccgccccattggcacccgttacctcacccgtaatctgtaa

SEQ ID NO: 22 - DNA, 7369 bp, synthetic construct
  source 1..7369: mol_type = other DNA
ccgccatgccggggttttacgagattgtgattaaggtccccagcgaccttgacgagcatctgcccggcatttctgacagctttgtgaactgggtggccgagaaggaatgggagttgccgccagattctgacatggatctgaatctgattgagcaggcacccctgaccgtggccgagaagctgcagcgcgactttctgacggaatggcgccgtgtgagtaaggccccggaggcccttttctttgtgcaatttgagaagggagagagctacttccacatgcacgtgctcgtggaaaccaccggggtgaaatccatggttttgggacgtttcctgagtcagattcgcgaaaaactgattcagagaatttaccgcgggatcgagccgactttgccaaactggttcgcggtcacaaagaccagaaatggcgccggaggcgggaacaaggtggtggatgagtgctacatccccaattacttgctccccaaaacccagcctgagctccagtgggcgtggactaatatggaacagtatttaagcgcctgtttgaatctcacggagcgtaaacggttggtggcgcagcatctgacgcacgtgtcgcagacgcaggagcagaacaaagagaatcagaatcccaattctgatgcgccggtgatcagatcaaaaacttcagccaggtacatggagctggtcgggtggctcgtggacaaggggattacctcggagaagcagtggatccaggaggaccaggcctcatacatctccttcaatgcggcctccaactcgcggtcccaaatcaaggctgccttggacaatgcgggaaagattatgagcctgactaaaaccgcccccgactacctggtgggccagcagcccgtggaggacatttccagcaatcggatttataaaattttggaactaaacgggtacgatccccaatatgcggcttccgtctttctgggatgggccacgaaaaagttcggcaagaggaacaccatctggctgtttgggcctgcaactaccgggaagaccaacatcgcggaggccatagcccacactgtgcccttctacgggtgcgtaaactggaccaatgagaactttcccttcaacgactgtgtcgacaagatggtgatctggtgggaggaggggaagatgaccgccaaggtcgtggagtcggccaaagccattctcggaggaagcaaggtgcgcgtggaccagaaatgcaagtcctcggcccagatagacccgactcccgtgatcgtcacctccaacaccaacatgtgcgccgtgattgacgggaactcaacgaccttcgaacaccagcagccgttgcaagaccggatgttcaaatttgaactcacccgccgtctggatcatgactttgggaaggtcaccaagcaggaagtcaaagactttttccggtgggcaaaggatcacgtggttgaggtggagcatgaattctacgtcaaaaagggtggagccaagaaaagacccgcccccagtgacgcagatataagtgagcccaaacgggtgcgcgagtcagttgcgcagccatcgacgtcagacgcggaagcttcgatcaactacgcagacaggtaccaaaacaaatgttctcgtcacgtgggcatgaatctgatgctgtttccctgcagacaatgcgagagaatgaatcagaattcaaatatctgcttcactcacggacagaaagactgtttagagtgctttcccgtgtcagaatctcaacccgtttctgtcgtcaaaaaggcgtatcagaaactgtgctacattcatcatatcatgggaaaggtgccagacgcttgcactgcctgcgatctggtcaatgtggatttggatgactgcatctttgaacaataaatgatttaaatcaggtatggctgccgatggttatcttccagattggctcgaggacactctctctgaaggaataagacagtggtggaagctcaaacctggcccaccaccaccaaagcccgcagagcggcataaggacgacagcaggggtcttgtgcttcctgggtacaagtacctcggacccttcaacggactcgacaagggagagccggtcaacgaggcagacgccgcggccctcgagcacgacaaagcctacgaccggcagctcgacagcggagacaacccgtacctcaagtacaaccacgccgacgccgagttccaggagcggctcaaagaagatacgtcttttgggggcaacctcgggcgagcagtcttccaggccaaaaagaggcttcttgaacctcttggtctggttgaggaagcggctaagacggctcctggaaagaagaggcctgtagagcactctcctgtggagccagactcctcctcgggaaccggaaaggcgggccagcagcctgcaagaaaaagattgaattttggtcagactggagacgcagactcagtcccagaccctcaaccaatcggagaacctcccgcagccccctcaggtgtgggatctcttacaatggctgcaggcggtggcgcaccaatggcagacaataacgagggcgccgacggagtgggtaattcctcgggaaattggcattgcgattccacatggatgggcgacagagtcatcaccaccagcacccgaacctgggccctgcccacctacaacaaccacctctacaagcaaatctccaacagcacatctggaggatcttcaaatgacaacgcctacttcggctacagcaccccctgggggtattttgactttaacagattccactgccacttttcaccacgtgactggcagcgactcatcaacaacaactggggattccggcccaagagactcagcttcaagctcttcaacatccaggtcaaggaggtcacgcagaatgaaggcaccaagaccatcgccaataacctcaccagcaccatccaggtgtttacggactcggagtaccagctgccgtacgttctcggctctgcccaccagggctgcctgcctccgttcccggcggacgtgttcatgattccccagtacggctacctaacactcaacaacggtagtcaggccgtgggacgctcctccttctactgcctggaatactttccttcgcagatgctgagaaccggcaacaacttccagtttacttacaccttcgaggacgtgcctttccacagcagctacgcccacagccagagcttggaccggctgatgaatcctctgattgaccagtacctgtactacttgtctcggactcaaacaacaggaggcacgacaaatacgcagactctgggcttcagccaaggtgggcctaatacaatggccaatcaggcaaagaactggctgccaggaccctgttaccgccagcagcgagtatcaaagacatctgcggataacaacaacagtgaatactcgtggactggagctaccaagtaccacctcaatggcagagactctctggtgaatccgggcccggccatggcaagccacaaggacgatgaagaaaagttttttcctcagagcggggttctcatctttgggaagcaaggctcagagaaaacaaatgtggacattgaaaaggtcatgattacagacgaagaggaaatcaggacaaccaatcccgtggctacggagcagtatggttctgtatctaccaacctccagagaggcaacgcagcagcaccacgtggtgatctggcaccagcagcaagacaagcagctaccgcagatgtcaacacacaaggcgttcttccaggcatggtctggcaggacagagatgtgtaccttcaggggcccatctgggcaaagattccacacacggacggacattttcacccctctcccctcatgggtggattcggacttaaacaccctccgcctcagatcctgatcaagaacacgcctgtacctgcggatcctccgaccaccttcaaccagtcaaagctgaactctttcatcacccagtattctactggccaagtcagcgtggagatcgagtgggagctgcagaaggaaaacagcaagcgctggaaccccgagatccagtacacctccaactactacaaatctacaagtgtggactttgctgttaatacagaaggcgtgtactctgaaccccgccccattggcacccgttacctcacccgtaatctgtaattgcctgttaatcaataaaccggttgattcgtttcagttgaactttggtctctgcgaagggcgaattcgtttaaacctgcaggactagaggtcctgtattagaggtcacgtgagtgttttgcgacattttgcgacaccatgtggtcacgctgggtatttaagcccgagtgagcacgcagggtctccattttgaagcgggaggtttgaacgcgcagccgccaagccgaattctgcagatatccatcacactggcggccgctcgactagagcggccgccaccgcggtggagctccagcttttgttccctttagtgagggttaattgcgcgcttggcgtaatcatggtcatagctgtttcctgtgtgaaattgttatccgctcacaattccacacaacatacgagccggaagcataaagtgtaaagcctggggtgcctaatgagtgagctaactcacattaattgcgttgcgctcactgcccgctttccagtcgggaaacctgtcgtgccagctgcattaatgaatcggccaacgcgcggggagaggcggtttgcgtattgggcgctcttccgcttcctcgctcactgactcgctgcgctcggtcgttcggctgcggcgagcggtatcagctcactcaaaggcggtaatacggttatccacagaatcaggggataacgcaggaaagaacatgtgagcaaaaggccagcaaaaggccaggaaccgtaaaaaggccgcgttgctggcgtttttccataggctccgcccccctgacgagcatcacaaaaatcgacgctcaagtcagaggtggcgaaacccgacaggactataaagataccaggcgtttccccctggaagctccctcgtgcgctctcctgttccgaccctgccgcttaccggatacctgtccgcctttctcccttcgggaagcgtggcgctttctcatagctcacgctgtaggtatctcagttcggtgtaggtcgttcgctccaagctgggctgtgtgcacgaaccccccgttcagcccgaccgctgcgccttatccggtaactatcgtcttgagtccaacccggtaagacacgacttatcgccactggcagcagccactggtaacaggattagcagagcgaggtatgtaggcggtgctacagagttcttgaagtggtggcctaactacggctacactagaagaacagtatttggtatctgcgctctgctgaagccagttaccttcggaaaaagagttggtagctcttgatccggcaaacaaaccaccgctggtagcggtggtttttttgtttgcaagcagcagattacgcgcagaaaaaaaggatctcaagaagatcctttgatcttttctacggggtctgacgctcagtggaacgaaaactcacgttaagggattttggtcatgagattatcaaaaaggatcttcacctagatccttttaaattaaaaatgaagttttaaatcaatctaaagtatatatgagtaaacttggtctgacagttaccaatgcttaatcagtgaggcacctatctcagcgatctgtctatttcgttcatccatagttgcctgactccccgtcgtgtagataactacgatacgggagggcttaccatctggccccagtgctgcaatgataccgcgagacccacgctcaccggctccagatttatcagcaataaaccagccagccggaagggccgagcgcagaagtggtcctgcaactttatccgcctccatccagtctattaattgttgccgggaagctagagtaagtagttcgccagttaatagtttgcgcaacgttgttgccattgctacaggcatcgtggtgtcacgctcgtcgtttggtatggcttcattcagctccggttcccaacgatcaaggcgagttacatgatcccccatgttgtgcaaaaaagcggttagctccttcggtcctccgatcgttgtcagaagtaagttggccgcagtgttatcactcatggttatggcagcactgcataattctcttactgtcatgccatccgtaagatgcttttctgtgactggtgagtactcaaccaagtcattctgagaatagtgtatgcggcgaccgagttgctcttgcccggcgtcaatacgggataataccgcgccacatagcagaactttaaaagtgctcatcattggaaaacgttcttcggggcgaaaactctcaaggatcttaccgctgttgagatccagttcgatgtaacccactcgtgcacccaactgatcttcagcatcttttactttcaccagcgtttctgggtgagcaaaaacaggaaggcaaaatgccgcaaaaaagggaataagggcgacacggaaatgttgaatactcatactcttcctttttcaatattattgaagcatttatcagggttattgtctcatgagcggatacatatttgaatgtatttagaaaaataaacaaataggggttccgcgcacatttccccgaaaagtgccacctaaattgtaagcgttaatattttgttaaaattcgcgttaaatttttgttaaatcagctcattttttaaccaataggccgaaatcggcaaaatcccttataaatcaaaagaatagaccgagatagggttgagtgttgttccagtttggaacaagagtccactattaaagaacgtggactccaacgtcaaagggcgaaaaaccgtctatcagggcgatggcccactacgtgaaccatcaccctaatcaagttttttggggtcgaggtgccgtaaagcactaaatcggaaccctaaagggagcccccgatttagagcttgacggggaaagccggcgaacgtggcgagaaaggaagggaagaaagcgaaaggagcgggcgctagggcgctggcaagtgtagcggtcacgctgcgcgtaaccaccacacccgccgcgcttaatgcgccgctacagggcgcgtcccattcgccattcaggctgcgcaactgttgggaagggcgatcggtgcgggcctcttcgctattacgccagctggcgaaagggggatgtgctgcaaggcgattaagttgggtaacgccagggttttcccagtcacgacgttgtaaaacgacggccagtgagcgcgcgtaatacgactcactatagggcgaattgggtaccgggccccccctcgatcgaggtcgacggtatcgggggagctcgcagggtctccattttgaagcgggaggtttgaacgcgcag

SEQ ID NO: 23 - DNA, 781 bp, synthetic construct
  source 1..781: mol_type = other DNA
ctccggagcttctattcctgatccctgcataagaaggagacatggtggtggtggtggtgggtgggggtggtggggcacagaggaagccggtactgggctctgcaccccattcccgctcccagatccctctggacacagcatttttctccagtgagcacagcctccccttgccccacagccaacagcaacatgcctcccaacaaaagcatctgtccctcagccaaaacccctgttgcctctctctggggaaattgtagggctgggccagggtggggggaccattctctgcagggagattaggagtgtctgtcaggggcgggtggagcggggtggggccctggcttactcacatccttgagagtcctttgctggcagatttggggagcccacagctcagatgtctgtctcagcattgtcttccaagctcctaggccacagtagtggggggctcccttctctggcttcttctttggtgacagtcaaggtggggttgggggtgacagagggtcctgcttctcttctaggagcagttgatcccaggaagagcattggagcctccagcaggggctgttggggcctgtctgaggagataggatgcgtcaggcagccccagacacgatcacattcctctcaacatgcctgccggggtctgtggagcctaggggctgatgggagggtggggtgggggccggaagggtttaggtctatataagcagagctcgtttagtgaaccgtcagtccgcctggagacctcgagccgagtggtcgtgcctccatagaa

SEQ ID NO: 24 - DNA, 5526 bp, synthetic construct
  source 1..5526: mol_type = other DNA
cttccgcttcctcgctcactgactcgctgcgctcggtcgttcggctgcggcgagcggtatcagctcactcaaaggcggtaatacggttatccacagaatcaggggataacgcaggaaagaacatgtgagcaaaaggccagcaaaaggccaggaaccgtaaaaaggccgcgttgctggcgtttttccataggctccgcccccctgacgagcatcacaaaaatcgacgctcaagtcagaggtggcgaaacccgacaggactataaagataccaggcgtttccccctggaagctccctcgtgcgctctcctgttccgaccctgccgcttaccggatacctgtccgcctttctcccttcgggaagcgtggcgctttctcatagctcacgctgtaggtatctcagttcggtgtaggtcgttcgctccaagctgggctgtgtgcacgaaccccccgttcagcccgaccgctgcgccttatccggtaactatcgtcttgagtccaacccggtaagacacgacttatcgccactggcagcagccactggtaacaggattagcagagcgaggtatgtaggcggtgctacagagttcttgaagtggtggcctaactacggctacactagaagaacagtatttggtatctgcgctctgctgaagccagttaccttcggaaaaagagttggtagctcttgatccggcaaacaaaccaccgctggtagcggtggtttttttgtttgcaagcagcagattacgcgcagaaaaaaaggatctcaagaagatcctttgatcttttctacggggtctgacgctcagtggaacgaaaactcacgttaagggattttggtcatgagattatcaaaaaggatcttcacctagatccttttaaattaaaaatgaagttttaaatcaatctaaagtatatatgagtaaacttggtctgacagttaccaatgcttaatcagtgaggcacctatctcagcgatctgtctatttcgttcatccatagttgcctgactccccgtcgtgtagataactacgatacgggagggcttaccatctggccccagtgctgcaatgataccgcgagacccacgctcaccggctccagatttatcagcaataaaccagccagccggaagggccgagcgcagaagtggtcctgcaactttatccgcctccatccagtctattaattgttgccgggaagctagagtaagtagttcgccagttaatagtttgcgcaacgttgttgccattgctacaggcatcgtggtgtcacgctcgtcgtttggtatggcttcattcagctccggttcccaacgatcaaggcgagttacatgatcccccatgttgtgcaaaaaagcggttagctccttcggtcctccgatcgttgtcagaagtaagttggccgcagtgttatcactcatggttatggcagcactgcataattctcttactgtcatgccatccgtaagatgcttttctgtgactggtgagtactcaaccaagtcattctgagaatagtgtatgcggcgaccgagttgctcttgcccggcgtcaatacgggataataccgcgccacatagcagaactttaaaagtgctcatcattggaaaacgttcttcggggcgaaaactctcaaggatcttaccgctgttgagatccagttcgatgtaacccactcgtgcacccaactgatcttcagcatcttttactttcaccagcgtttctgggtgagcaaaaacaggaaggcaaaatgccgcaaaaaagggaataagggcgacacggaaatgttgaatactcatactcttcctttttcaatattattgaagcatttatcagggttattgtctcatgagcggatacatatttgaatgtatttagaaaaataaacaaataggggttccgcgcacatttccccgaaaagtgccacctaaattgtaagcgttaatattttgttaaaattcgcgttaaatttttgttaaatcagctcattttttaaccaataggccgaaatcggcaaaatcccttataaatcaaaagaatagaccgagatagggttgagtgttgttccagtttggaacaagagtccactattaaagaacgtggactccaacgtcaaagggcgaaaaaccgtctatcagggcgatggcccactacgtgaaccatcaccctaatcaagttttttggggtcgaggtgccgtaaagcactaaatcggaaccctaaagggagcccccgatttagagcttgacggggaaagccggcgaacgtggcgagaaaggaagggaagaaagcgaaaggagcgggcgctagggcgctggcaagtgtagcggtcacgctgcgcgtaaccaccacacccgccgcgcttaatgcgccgctacagggcgcgtcccattcgccattcaggctgcgcaactgttgggaagggcgatcggtgcgggcctcttcgctattacgccagctgcgcgctcgctcgctcactgaggccgcccgggcaaagcccgggcgtcgggcgacctttggtcgcccggcctcagtgagcgagcgagcgcgcagagagggagtggccaactccatcactaggggttccttgtagttaatgattaacccgccatgctacttatctacgtagccatgctctaggaagagtaccattgacgtcaataatgacgtatgttcccatagtaacgccaatagggactttccattgacgtcaatgggtggagtatttacggtaaactgcccacttggcagtacatcaagtgtatcatatgctccggagcttctattcctgatccctgcataagaaggagacatggtggtggtggtggtgggtgggggtggtggggcacagaggaagccggtactgggctctgcaccccattcccgctcccagatccctctggacacagcatttttctccagtgagcacagcctccccttgccccacagccaacagcaacatgcctcccaacaaaagcatctgtccctcagccaaaacccctgttgcctctctctggggaaattgtagggctgggccagggtggggggaccattctctgcagggagattaggagtgtctgtcaggggcgggtggagcggggtggggccctggcttactcacatccttgagagtcctttgctggcagatttggggagcccacagctcagatgtctgtctcagcattgtcttccaagctcctaggccacagtagtggggggctcccttctctggcttcttctttggtgacagtcaaggtggggttgggggtgacagagggtcctgcttctcttctaggagcagttgatcccaggaagagcattggagcctccagcaggggctgttggggcctgtctgaggagataggatgcgtcaggcagccccagacacgatcacattcctctcaacatgcctgccggggtctgtggagcctaggggctgatgggagggtggggtgggggccggaagggtttaggtctatataagcagagctcgtttagtgaaccgtcagtccgcctggagacctcgagccgagtggtcgtgcctccatagaaggatccgccaccatggtgagcaagggcgaggagctgttcaccggggtggtgcccatcctggtcgagctggacggcgacgtaaacggccacaagttcagcgtgtccggcgagggcgagggcgatgccacctacggcaagctgaccctgaagttcatttgcaccaccggcaagctgcccgtgccctggcccaccctcgtgaccaccctgacctacggcgtgcagtgcttcagccgctaccccgaccacatgaagcagcacgacttcttcaagtccgccatgcccgaaggctacgtccaggagcgcaccatcttcttcaaggacgacggcaactacaagacccgcgccgaggtgaagttcgagggcgacaccctggtgaaccgcatcgagctgaagggcatcgacttcaaggaggacggcaacatcctggggcacaagctggagtacaactacaacagccacaacgtctatatcatggccgacaagcagaagaacggcatcaaggtgaacttcaagatccgccacaacatcgaggacggcagcgtgcagctcgccgaccactaccagcagaacacccccatcggcgacggccccgtgctgctgcccgacaaccactacctgagcacccagtccgccctgagcaaagaccccaacgagaagcgcgatcacatggtcctgctggagttcgtgaccgccgccgggatcactctcggcatggacgagctgtacaagtccggactcagatctgatccaaaaaagaagagaaaggtagatccaaaaaagaagagaaaggtagatccaaaaaagaagagaaaggtataaaagcttcgaggaattcgaagcttctaggtaccgaattcgatatcaagcttatcgataatcaacctctggattacaaaatttgtgaaagattgactggtattcttaactatgttgctccttttacgctatgtggatacgctgctttaatgcctttgtatcatgctattgcttcccgtatggctttcattttctcctccttgtataaatcctggttgctgtctctttatgaggagttgtggcccgttgtcaggcaacgtggcgtggtgtgcactgtgtttgctgacgcaacccccactggttggggcattgccaccacctgtcagctcctttccgggactttcgctttccccctccctattgccacggcggaactcatcgccgcctgccttgcccgctgctggacaggggctcggctgttgggcactgacaattccgtggtgttgtcggggaaatcatcgtcctttccttggctgctcgcctgtgttgccacctggattctgcgcgggacgtccttctgctacgtcccttcggccctcaatccagcggaccttccttcccgcggcctgctgccggctctgcggcctcttccgcgtcttcgccttcgccctcagacgagtcggatctccctttgggccgcctccccgcatcgataccgtcgacccgggcggccgcttcgagcagacatgataagatacattgatgagtttggacaaaccacaactagaatgcagtgaaaaaaatgctttatttgtgaaatttgtgatgctattgctttatttgtaaccattataagctgcaataaacaagttaacaacaacaattgcattcattttatgtttcaggttcagggggagatgtgggaggttttttaaagcaagtaaaacctctacaaatgtggtaaaatcgataaggatcttcctagagcatggctacgtagataagtagcatggcgggttaatcattaactacaaggaacccctagtgatggagttggccactccctctctgcgcgctcgctcgctcactgaggccgggcgaccaaaggtcgcccgacgcccgggctttgcccgggcggcctcagtgagcgagcgagcgcgcagctgcattaatgaatcggccaacgcgcggggagaggcggtttgcgtattgggcgct

SEQ ID NO: 25 - DNA, 776 bp, synthetic construct
  source 1..776: mol_type = other DNA
ctccggagcttctattcctgatccctgcagaagaaggagacggtggtggtggtgggtgggggtggcagggcacagaggaagccagtaccgggccctgcaccccattcccactcccagatccctctggacacagcatttttctccagtgagcacagccttcccttgccccacagccaacagcaacatggctcccaacaaaagcatctgcccctcagccaaaacccctgttgcctctctctggggaaattgtaggactgggtcagggtgggggaaccattctctgcagggagattaggagtgtctgtcaggggtgggtggagcggggtggggccctggcttactcacatcctcgagagtcctttgctggcagatttggggagcccacagcacaggtgtctgtctcagtattgtcttccaagctcctaggccacagtagtggggggctcccctctctggctttttctttggtgacagtcaaggttgggggtggggtgagagagggtcctgcttttcttctaggaacagttgatcccaggaagagcagtggagcctccagcaggggctgttggggcctgtctgaggagataggacgcgtcaggcagccccagacacgaccacattcctcccaacatgcctgccggggtctgtggagcccaggggctgaggggagggtggggtgggggccggaagggtttaggtctatataagcagagctcgtttagtgaaccgtcagtccgcctggagacctcgagccgagtggtcgtgcctccatagaa

SEQ ID NO: 26 - DNA, 1004 bp, Homo sapiens
  source 1..1004: mol_type = genomic DNA
ctccggagcttctattcctgatccctgcagaagaaggagacggtggtggtggtgggtgggggtggcagggcacagaggaagccagtaccgggccctgcaccccattcccactcccagatccctctggacacagcatttttctccagtgagcacagccttcccttgccccacagccaacagcaacatggctcccaacaaaagcatctgcccctcagccaaaacccctgttgcctctctctggggaaattgtaggactgggtcagggtgggggaaccattctctgcagggagattaggagtgtctgtcaggggtgggtggagcggggtggggccctggcttactcacatcctcgagagtcctttgctggcagatttggggagcccacagcacaggtgtctgtctcagtattgtcttccaagctcctaggccacagtagtggggggctcccctctctggctttttctttggtgacagtcaaggttgggggtggggtgagagagggtcctgcttttcttctaggaacagttgatcccaggaagagcagtggagcctccagcaggggctgttggggcctgtctgaggagataggacgcgtcaggcagccccagacacgaccacattcctcccaacatgcctgccggggtctgtggagcccaggggctgaggggagggtggggtgggggccggaagggtttgagggctgggactcccggggccccatgggaaagtgtagcctgcaggcccatacctccccctgtgaatcacgcctggcgggacaagaaagcccaaaataccccaaacaatgagtttccagtaaaatatgacagacatgatgaggtggaggagaggagggacctggctgggagttggcgctagcctgtgggtgatgaaagccaaggggaatggaaagtgccaggcccgcctcctacccatgagtataaagcactcgcatccctttccaatttacccgagcaccttctcttcactcagccaactgctcgctc

SEQ ID NO: 27 - DNA, 2002 bp, Homo sapiens
  source 1..2002: mol_type = genomic DNA
ctccggagcttctattcctgatccctgcataagaaggagacatggtggtggtggtggtgggtgggggtggtggggcacagaggaagccggtactgggctctgcaccccattcccgctcccagatccctctggacacagcatttttctccagtgagcacagcctccccttgccccacagccaacagcaacatgcctcccaacaaaagcatctgtccctcagccaaaacccctgttgcctctctctggggaaattgtagggctgggccagggtggggggaccattctctgcagggagattaggagtgtctgtcaggggcgggtggagcggggtggggccctggcttactcacatccttgagagtcctttgctggcagatttggggagcccacagctcagatgtctgtctcagcattgtcttccaagctcctaggccacagtagtggggggctcccttctctggcttcttctttggtgacagtcaaggtggggttgggggtgacagagggtcctgcttctcttctaggagcagttgatcccaggaagagcattggagcctccagcaggggctgttggggcctgtctgaggagataggatgcgtcaggcagccccagacacgatcacattcctctcaacatgcctgccggggtctgtggagcctaggggctgatgggagggtggggtgggggccggaagggtttgctttgggaggttgtctgggagattgctgaagttttgatatacacacctccaaagcaggaccaagtggactcctagaaatgtcccctgacccttggggcttcaggagtcagggaccctcgtgtccacctcagccttgcccttggcacagcccagctccactccagcctctactcctccccagaacatctcctgggccagttccacaaggggctcaaacgagggcgcctgagctgcccacactagggatgttctgggggtctgagaagatatctggggctggaagaataaaaggcccccctaggcctgttcctggatgcagctccagccactttggggctaagcctgggctataacaatgccaacgaggcttcttgccatactcggtttacaaaaccctttcacatacattgtcgcattggattctcagagctgactgcactaagcagaatagatggtatgactcccactttgcagatgagaacactgaggctcagagaagtgccaagccctgggtcacagaggcgtaaatggcagagccaggacccacctgactccaggctgtttcctggcctccatgaggccacctgccctatggtgtggtggatgtgagatcctcaccatagggaggagattagggtctgtgctcagggatggggagagctgcctggatttctctttgatggggatgttggggtgggaatcacgatacacctgactagctgggtgtatttcagggatgggacagacttctcagcacagcatgggaggtcaggcctgggagggccccccagacctccttgtctctaatagagggtcatggtgagggaggcctgtctgtgcccaaggtgaccttgccatgccggtgctttccagccgggtatccatcccctgcagcagcaggcttcctctacgtggatgttaaaggcccattcagttcatggagagctagcaggtaactaggtttaaggtgcagaggccctgctctctgtcaccctggctaagcccagtgcgcgggttcctgagggctgggactcccagggtccgatgggaaagtgtagcctgcaggcccacacctccccctgtgaatcacgcctggcgggacaagaaagcccaaaacactccaaacaatgagtttccagtaaaatatgacagacatgatgaggcggatgagaggagggacctggctgggagttggcgctagcctgtgggtgatgaaagccaaggggaatggaaagtgccagacccgccccctacccacgagtataaagcactcgcatccctttccaatttacccgagcacc

SEQ ID NO: 28 - DNA, 1010 bp, Homo sapiens
  source 1..1010: mol_type = genomic DNA
ctccggagcttctattcctgatccctgcataagaaggagacatggtggtggtggtggtgggtgggggtggtggggcacagaggaagccggtactgggctctgcaccccattcccgctcccagatccctctggacacagcatttttctccagtgagcacagcctccccttgccccacagccaacagcaacatgcctcccaacaaaagcatctgtccctcagccaaaacccctgttgcctctctctggggaaattgtagggctgggccagggtggggggaccattctctgcagggagattaggagtgtctgtcaggggcgggtggagcggggtggggccctggcttactcacatccttgagagtcctttgctggcagatttggggagcccacagctcagatgtctgtctcagcattgtcttccaagctcctaggccacagtagtggggggctcccttctctggcttcttctttggtgacagtcaaggtggggttgggggtgacagagggtcctgcttctcttctaggagcagttgatcccaggaagagcattggagcctccagcaggggctgttggggcctgtctgaggagataggatgcgtcaggcagccccagacacgatcacattcctctcaacatgcctgccggggtctgtggagcctaggggctgatgggagggtggggtgggggccggaagggtttgagggctgggactcccagggtccgatgggaaagtgtagcctgcaggcccacacctccccctgtgaatcacgcctggcgggacaagaaagcccaaaacactccaaacaatgagtttccagtaaaatatgacagacatgatgaggcggatgagaggagggacctggctgggagttggcgctagcctgtgggtgatgaaagccaaggggaatggaaagtgccagacccgccccctacccacgagtataaagcactcgcatccctttccaatttacccgagcaccttctcttcactcagccaactgctcgctcg

SEQ ID NO: 29 - DNA, 2005 bp, Homo sapiens
  source 1..2005: mol_type = genomic DNA
ctccggagcttctattcctgatccctgcagaagaaggagacggtggtggtggtgggtgggggtggcagggcacagaggaagccagtaccgggccctgcaccccattcccactcccagatccctctggacacagcatttttctccagtgagcacagccttcccttgccccacagccaacagcaacatggctcccaacaaaagcatctgcccctcagccaaaacccctgttgcctctctctggggaaattgtaggactgggtcagggtgggggaaccattctctgcagggagattaggagtgtctgtcaggggtgggtggagcggggtggggccctggcttactcacatcctcgagagtcctttgctggcagatttggggagcccacagcacaggtgtctgtctcagtattgtcttccaagctcctaggccacagtagtggggggctcccctctctggctttttctttggtgacagtcaaggttgggggtggggtgagagagggtcctgcttttcttctaggaacagttgatcccaggaagagcagtggagcctccagcaggggctgttggggcctgtctgaggagataggacgcgtcaggcagccccagacacgaccacattcctcccaacatgcctgccggggtctgtggagcccaggggctgaggggagggtggggtgggggccggaagggtttgctttgggaggttgtctgggagattgctgaagttttgatatacacacctccaaagcaggaccaagtggactcctagaaatgtcccctgacccttggggcttcaggagtcagggacccttgtgtccacttcagccttgcccttggcacagcctggcaccactccagcttctactcctccccagaacatctcctgggccagttccacaaggggctcaaacgagggcacctgagccagacttctgcctacactagggatgttctgggggtctgagaggatatctggggctggaagaaaaaaaggcccccctaggcctgttcctggatgcagctccatccactttggggctaagcctgggctacaacaatgccaaccaggcttcttgccatactcggtttacaaaagcctttcacatacgctgtcgcattggcttctcacagctgactgcagtaggcagagtagatggtatgactcccactttgcagatgagaacactgaggctcagagaagcgccaagccctgggtcacgggggcgtaaatggcagagccaggacccacctgactccaggctgtttcctggcctccatgaggccacccgccctatggtgtggtggatgtcagatcctcaccgtagggaggaaattagggtctgtgcccggggctggggagagctgcctagatttctctttgatgggggtgttggggtgggaatcaccatacacctgactggctgagtgtatttcagggatgggacaggcttctcagcacagcatggcaggtcaggcctgggagggccccccagacctccttgtctctaacagcgggtcatggtgagggaggcctctctgtgcccaaggtgaccttgccatgccggtgctctccagctgggtatctgtcccctgcagtggtgggcttcctctaagtggatggtaaaggcccatccagttcatggagagctagcaggtcaccaggtttaaggtgcagaggccctgctctctgtcaccctggctgagcccagtgtgcgggttcctgagggctgggactcccggggccccatgggaaagtgtagcctgcaggcccatacctccccctgtgaatcacgcctggcgggacaagaaagcccaaaataccccaaacaatgagtttccagtaaaatatgacagacatgatgaggtggaggagaggagggacctggctgggagttggcgctagcctgtgggtgatgaaagccaaggggaatggaaagtgccaggcccgcctcctacccatgagtataaagcactcgcatccctttccaatttacccgagcacc

SEQ ID NO: 30 - DNA, 5526 bp, synthetic construct; identical to SEQ ID NO: 8
  source 1..5526: mol_type = other DNA

SEQ ID NO: 31 - DNA, 5547 bp, synthetic construct; identical to SEQ ID NO: 9
  source 1..5547: mol_type = other DNA